European Patent Application EP 4 397 681 A1, published July 10, 2024. Title: ANTIBODY, IMMOBILIZED ANTIBODY USING THE SAME, ANTIBODY COMPOSITION, REAGENT FOR IMMUNOASSAY AND IMMUNOASSAY METHOD, AS WELL AS METHOD FOR IMPROVING REACTIVITY OF ANTIBODY WITH ANTIGEN. Applicant: EIKEN KAGAKU KABUSHIKI KAISHA. Application JP. The sequence listing filed with the application follows.

SEQUENCE LISTING (4 sequences)

SEQ ID NO: 1 - DNA, 26 bp, synthetic construct
  source 1..26: mol_type = other DNA; note = N297S-primerF
cagttcagcagcactttccgctcagt

SEQ ID NO: 2 - DNA, 26 bp, synthetic construct
  source 1..26: mol_type = other DNA; note = N297S-primerR
agtgctgctgaactgctcctcccggg

SEQ ID NO: 3 - DNA, 28 bp, synthetic construct
  source 1..28: mol_type = other DNA; note = N297C-S298C-primerF
cagttctgctgcactttccgctcagtca

SEQ ID NO: 4 - DNA, 28 bp, synthetic construct
  source 1..28: mol_type = other DNA; note = N297C-S298C-primerR
aagtgcagcagaactgctcctcccgggg